European Patent Specification EP 3 967 703 B1, published July 26, 2023. Title: CYCLIC PEPTIDE, SCAFFOLD MATERIAL FOR CELL, CELL ISOLATION. Applicant: FUJIFILM Corporation. The sequence listing filed with the application follows.

SEQUENCE LISTING (49 sequences)

SEQ ID NO: 1 - protein, 11 aa, Artificial Sequence
  Integrin-binding Cyclic Peptide 1
  THIOETH (1)..(8): Thioether bridge between residues 1 and 8
  MISC_FEATURE (1)..(1): N- alpha-acetyl- isoleucine
  THIOETH (2)..(6): Thioether bridge between residues 2 and 6
  MISC_FEATURE (2)..(2): 2-amino-3-(acetylamino)propanoic acid
  MISC_FEATURE (6)..(6): Homocystein
  MISC_FEATURE (8)..(8): Homocystein
XXRGDXFXKKK

SEQ ID NO: 2 - protein, 11 aa, Artificial Sequence
  Integrin-binding Cyclic Peptide 2
  THIOETH (1)..(8): Thioether bridge between residues 1 and 8
  MISC_FEATURE (1)..(1): N- alpha-acetyl- isoleucine
  MISC_FEATURE (2)..(2): 2-amino-4-(acetylamino)butanoic acid
  THIOETH (2)..(6): Thioether bridge between residues 2 and 6
  MISC_FEATURE (6)..(6): Homocystein
  MISC_FEATURE (8)..(8): Homocystein
XXRGDXFXKKK

SEQ ID NO: 3 - protein, 11 aa, Artificial Sequence
  Integrin-binding Cyclic Peptide 3
  THIOETH (1)..(8): Thioether bridge between residues 1 and 8
  MISC_FEATURE (1)..(1): N- alpha-acetyl- isoleucine
  MISC_FEATURE (2)..(2): N-delta-acetyl-ornithine
  THIOETH (2)..(6): Thioether bridge between residues 2 and 6
  MISC_FEATURE (6)..(6): Homocystein
  MISC_FEATURE (8)..(8): Homocystein
XXRGDXFXKKK

SEQ ID NO: 4 - protein, 11 aa, Artificial Sequence
  Integrin-binding Cyclic Peptide 4
  THIOETH (1)..(8): Thioether bridge between residues 1 and 8
  MISC_FEATURE (1)..(1): N- alpha-acetyl- isoleucine
  MISC_FEATURE (2)..(2): N-epsilon-acetyl-lysine
  THIOETH (2)..(6): Thioether bridge between residues 2 and 6
  MISC_FEATURE (6)..(6): Homocystein
  MISC_FEATURE (8)..(8): Homocystein
XXRGDXFXKKK

SEQ ID NO: 5 - protein, 11 aa, Artificial Sequence
  Integrin-binding Cyclic Peptide 5
  THIOETH (1)..(8): Thioether bridge between residues 1 and 8
  MISC_FEATURE (1)..(1): N- alpha-acetyl- isoleucine
  MISC_FEATURE (2)..(2): Homocystein
  THIOETH (2)..(6): Thioether bridge between residues 2 and 6
  MISC_FEATURE (6)..(6): 2-amino-3-(acetylamino)propanoic acid
  MISC_FEATURE (8)..(8): Homocystein
XXRGDXFXKKK

SEQ ID NO: 6 - protein, 11 aa, Artificial Sequence
  Integrin-binding Cyclic Peptide 6
  THIOETH (1)..(8): Thioether bridge between residues 1 and 8
  MISC_FEATURE (1)..(1): N- alpha-acetyl- isoleucine
  THIOETH (2)..(6): Thioether bridge between residues 2 and 6
  MISC_FEATURE (6)..(6): 2-amino-3-(acetylamino)propanoic acid
XCRGDXFCKKK

SEQ ID NO: 7 - protein, 11 aa, Artificial Sequence
  Integrin-binding Cyclic Peptide 7
  THIOETH (1)..(8): Thioether bridge between residues 1 and 8
  MISC_FEATURE (1)..(1): N- alpha-acetyl- isoleucine
  MISC_FEATURE (2)..(2): Homocystein
  THIOETH (2)..(6): Thioether bridge between residues 2 and 6
  MISC_FEATURE (6)..(6): 2-amino-4-(acetylamino)butanoic acid
  MISC_FEATURE (8)..(8): Homocystein
XXRGDXFXKKK

SEQ ID NO: 8 - protein, 11 aa, Artificial Sequence
  Integrin-binding Cyclic Peptide 8
  THIOETH (1)..(8): Thioether bridge between residues 1 and 8
  MISC_FEATURE (1)..(1): N- alpha-acetyl- isoleucine
  THIOETH (2)..(6): Thioether bridge between residues 2  and 6
  MISC_FEATURE (6)..(6): 2-amino-4-(acetylamino)butanoic acid
XCRGDXFCKKK

SEQ ID NO: 9 - protein, 11 aa, Artificial Sequence
  Integrin-binding Cyclic Peptide 9
  THIOETH (1)..(8): Thioether bridge between residues 1 and 8
  MISC_FEATURE (1)..(1): N- alpha-acetyl- isoleucine
  MISC_FEATURE (2)..(2): Homocystein
  THIOETH (2)..(6): Thioether bridge between residues 2 and 6
  MISC_FEATURE (6)..(6): N-delta-acetyl-ornithine
  MISC_FEATURE (8)..(8): Homocystein
XXRGDXFXKKK

SEQ ID NO: 10 - protein, 11 aa, Artificial Sequence
  Integrin-binding Cyclic Peptide 10
  THIOETH (1)..(8): Thioether bridge between residues 1 and 8
  MISC_FEATURE (1)..(1): N- alpha-acetyl- isoleucine
  THIOETH (2)..(6): Thioether bridge between residues 2 and 6
  MISC_FEATURE (6)..(6): N-delta-acetyl-ornithine
XCRGDXFCKKK

SEQ ID NO: 11 - protein, 11 aa, Artificial Sequence
  Integrin-binding Cyclic Peptide 11
  THIOETH (1)..(8): Thioether bridge between residues 1 and 8
  MISC_FEATURE (1)..(1): N- alpha-acetyl- isoleucine
  MISC_FEATURE (2)..(2): Homocystein
  THIOETH (2)..(6): Thioether bridge between residues 2 and 6
  MISC_FEATURE (6)..(6): N-epsilon-acetyl-lysine
  MISC_FEATURE (8)..(8): Homocystein
XXRGDXFXKKK

SEQ ID NO: 12 - protein, 11 aa, Artificial Sequence
  Integrin-binding Cyclic Peptide 12
  THIOETH (1)..(8): Thioether bridge between residues 1 and 8
  MISC_FEATURE (1)..(1): N- alpha-acetyl- isoleucine
  THIOETH (2)..(6): Thioether bridge between residues 2 and 6
  MISC_FEATURE (6)..(6): N-epsilon-acetyl-lysine
XCRGDXFCKKK

SEQ ID NO: 13 - protein, 11 aa, Artificial Sequence
  Integrin-binding Cyclic Peptide 13
  THIOETH (1)..(8): Thioether bridge between residues 1 and 8
  MISC_FEATURE (1)..(1): N- alpha-acetyl- isoleucine
  MISC_FEATURE (2)..(2): 2-amino-3-(acetylamino)propanoic acid
  THIOETH (2)..(6): Thioether bridge between residues 2 and 6
  MISC_FEATURE (6)..(6): Homocystein
XXRGDXFCKKK

SEQ ID NO: 14 - protein, 11 aa, Artificial Sequence
  Integrin-binding Cyclic Peptide 14
  THIOETH (1)..(8): Thioether bridge between residues 1 and 8
  MISC_FEATURE (1)..(1): N- alpha-acetyl- isoleucine
  MISC_FEATURE (2)..(2): 2-amino-3-(acetylamino)propanoic acid
  THIOETH (2)..(6): Thioether bridge between residues 2 and 6
  MISC_FEATURE (8)..(8): Homocystein
XXRGDCFXKKK

SEQ ID NO: 15 - protein, 11 aa, Artificial Sequence
  Integrin-binding Cyclic Peptide 15
  THIOETH (1)..(8): Thioether bridge between residues 1 and 8
  MISC_FEATURE (1)..(1): N- alpha-acetyl- isoleucine
  MISC_FEATURE (2)..(2): N-delta-acetyl-ornithine
  THIOETH (2)..(6): Thioether bridge between residues 2 and 6
  MISC_FEATURE (6)..(6): Homocystein
XXRGDXFCKKK

SEQ ID NO: 16 - protein, 11 aa, Artificial Sequence
  Integrin-binding Cyclic Peptide 16
  THIOETH (1)..(8): Thioether bridge between residues 1 and 8
  MISC_FEATURE (1)..(1): N- alpha-acetyl- isoleucine
  THIOETH (2)..(6): Thioether bridge between residues 2 and 6
  MISC_FEATURE (2)..(2): N-delta-acetyl-ornithine
  MISC_FEATURE (8)..(8): Homocystein
XXRGDCFXKKK

SEQ ID NO: 17 - protein, 11 aa, Artificial Sequence
  Integrin-binding Cyclic Peptide 17
  THIOETH (1)..(8): Thioether bridge between residues 1 and 8
  MISC_FEATURE (1)..(1): N- alpha-acetyl- isoleucine
  MISC_FEATURE (2)..(2): Homocystein
  THIOETH (2)..(6): Thioether bridge between residues 2 and 6
  MISC_FEATURE (6)..(6): N-epsilon-acetyl-lysine
XXRGDXFCKKK

SEQ ID NO: 18 - protein, 11 aa, Artificial Sequence
  Integrin-binding Cyclic Peptide 18
  THIOETH (1)..(8): Thioether bridge between residues 1 and 8
  MISC_FEATURE (1)..(1): N- alpha-acetyl- isoleucine
  THIOETH (2)..(6): Thioether bridge between residues 2 and 6
  MISC_FEATURE (6)..(6): N-epsilon-acetyl-lysine
  MISC_FEATURE (8)..(8): Homocystein
XCRGDXFXKKK

SEQ ID NO: 19 - protein, 11 aa, Artificial Sequence
  Integrin-binding Cyclic Peptide 19
  THIOETH (1)..(8): Thioether bridge between residues 1 and 8
  MISC_FEATURE (1)..(1): N- alpha-acetyl- isoleucine
  MISC_FEATURE (2)..(2): Homocystein
  THIOETH (2)..(6): Thioether bridge between residues 2 and 6
  MISC_FEATURE (6)..(6): 2-amino-4-(acetylamino)butanoic acid
XXRGDXFCKKK

SEQ ID NO: 20 - protein, 11 aa, Artificial Sequence
  Integrin-binding Cyclic Peptide 20
  THIOETH (1)..(8): Thioether bridge between residues 1 and 8
  MISC_FEATURE (1)..(1): N- alpha-acetyl- isoleucine
  THIOETH (2)..(6): Thioether bridge between residues 2 and 6
  MISC_FEATURE (6)..(6): 2-amino-4-(acetylamino)butanoic acid
  MISC_FEATURE (8)..(8): Homocystein
XCRGDXFXKKK

SEQ ID NO: 21 - protein, 11 aa, Artificial Sequence
  Integrin-binding Cyclic Peptide 21
  THIOETH (1)..(8): Thioether bridge between residues 1 and 8
  MISC_FEATURE (1)..(1): N-epsilon-acetyl-lysine
  MISC_FEATURE (2)..(2): 2-amino-3-(acetylamino)propanoic acid
  THIOETH (2)..(6): Thioether bridge between residues 2 and 6
  MISC_FEATURE (6)..(6): Homocystein
  MISC_FEATURE (8)..(8): Homocystein
XXRGDXFXKKK

SEQ ID NO: 22 - protein, 9 aa, Artificial Sequence
  Integrin-binding Cyclic Peptide 22
  THIOETH (1)..(8): Thioether bridge between residues 1 and 8
  MISC_FEATURE (1)..(1): N- alpha-acetyl- isoleucine
  THIOETH (2)..(6): Thioether bridge between residues 2 and 8
  MISC_FEATURE (2)..(2): Homocystein
  MISC_FEATURE (6)..(6): N-epsilon-acetyl-lysine
  MISC_FEATURE (8)..(8): Homocystein
XXRGDXFXK

SEQ ID NO: 23 - protein, 11 aa, Artificial Sequence
  Integrin-binding Cyclic Peptide 23
  THIOETH (1)..(8): Thioether bridge between residues 1 and 8
  MISC_FEATURE (1)..(1): N-Acetyl-L-isoleucine
  MISC_FEATURE (2)..(2): N-delta-acetyl-ornithine
  THIOETH (2)..(6): Thioether bridge between residues 2 and 6
  MISC_FEATURE (6)..(6): Homocystein
  MISC_FEATURE (8)..(8): penicillamine
XXRGDXFXKKK

SEQ ID NO: 24 - protein, 11 aa, Artificial Sequence
  Integrin-binding Cyclic Peptide 24
  THIOETH (1)..(8): Thioether bridge between residues 1 and 8
  MISC_FEATURE (1)..(1): N-Acetyl-L-Glutamine
  MISC_FEATURE (2)..(2): N-delta-acetyl-ornithine
  THIOETH (2)..(6): Thioether bridge between residues 2 and 6
  MISC_FEATURE (6)..(6): Homocystein
  MISC_FEATURE (8)..(8): penicillamine
XXRGDXFXKKK

SEQ ID NO: 25 - protein, 11 aa, Artificial Sequence
  Integrin-binding Cyclic Peptide 25
  THIOETH (1)..(8): Thioether bridge between residues 1 and 8
  MISC_FEATURE (1)..(1): N- alpha-acetyl- tyrosine
  THIOETH (2)..(6): Thioether bridge between residues 2 and 8
  MISC_FEATURE (2)..(2): Homocystein
  MISC_FEATURE (6)..(6): N-epsilon-acetyl-lysine
  MISC_FEATURE (8)..(8): Homocystein
XXRGDXFXKKK

SEQ ID NO: 26 - protein, 11 aa, Artificial Sequence
  Integrin-binding Cyclic Peptide 26
  THIOETH (1)..(8): Thioether bridge between residues 1 and 8
  MISC_FEATURE (1)..(1): N- alpha-acetyl- lysine
  THIOETH (2)..(6): Thioether bridge between residues 2 and 8
  MISC_FEATURE (2)..(2): Homocystein
  MISC_FEATURE (6)..(6): N-epsilon-acetyl-lysine
  MISC_FEATURE (8)..(8): Homocystein
XXRGDXFXKKK

SEQ ID NO: 27 - protein, 11 aa, Artificial Sequence
  Integrin-binding Cyclic Peptide 27
  THIOETH (1)..(8): Thioether bridge between residues 1 and 8
  MISC_FEATURE (1)..(1): N- alpha-acetyl- threonine
  THIOETH (2)..(6): Thioether bridge between residues 2 and 8
  MISC_FEATURE (2)..(2): Homocystein
  MISC_FEATURE (6)..(6): N-epsilon-acetyl-lysine
  MISC_FEATURE (8)..(8): Homocystein
XXRGDXFXKKK

SEQ ID NO: 28 - protein, 11 aa, Artificial Sequence
  Integrin-binding Cyclic Peptide 28
  THIOETH (1)..(8): Thioether bridge between residues 1 and 8
  MISC_FEATURE (1)..(1): N- alpha-acetyl- valine
  THIOETH (2)..(6): Thioether bridge between residues 2 and 8
  MISC_FEATURE (2)..(2): Homocystein
  MISC_FEATURE (6)..(6): N-epsilon-acetyl-lysine
  MISC_FEATURE (8)..(8): Homocystein
XXRGDXFXKKK

SEQ ID NO: 29 - protein, 11 aa, Artificial Sequence
  Integrin-binding Cyclic Peptide 29
  THIOETH (1)..(8): Thioether bridge between residues 1 and 8
  MISC_FEATURE (1)..(1): N- alpha-acetyl- aspartic acid
  THIOETH (2)..(6): Thioether bridge between residues 2 and 8
  MISC_FEATURE (2)..(2): Homocystein
  MISC_FEATURE (6)..(6): N-epsilon-acetyl-lysine
  MISC_FEATURE (8)..(8): Homocystein
XXRGDXFXKKK

SEQ ID NO: 30 - protein, 11 aa, Artificial Sequence
  Integrin-binding Cyclic Peptide 30
  THIOETH (1)..(8): Thioether bridge between residues 1 and 8
  MISC_FEATURE (1)..(1): N- alpha-acetyl- glutamic acid
  THIOETH (2)..(6): Thioether bridge between residues 2 and 8
  MISC_FEATURE (2)..(2): Homocystein
  MISC_FEATURE (6)..(6): N-epsilon-acetyl-lysine
  MISC_FEATURE (8)..(8): Homocystein
XXRGDXFXKKK

SEQ ID NO: 31 - protein, 11 aa, Artificial Sequence
  Integrin-binding Cyclic Peptide 31
  THIOETH (1)..(8): Thioether bridge between residues 1 and 8
  MISC_FEATURE (1)..(1): N- alpha-acetyl- isoleusine
  THIOETH (2)..(6): Thioether bridge between residues 2 and 8
  MISC_FEATURE (2)..(2): Homocystein
  MISC_FEATURE (6)..(6): N-epsilon-acetyl-lysine
  MISC_FEATURE (8)..(8): Homocystein
XXRGDXPXKKK

SEQ ID NO: 32 - protein, 11 aa, Artificial Sequence
  Integrin-binding Cyclic Peptide 32
  THIOETH (1)..(8): Thioether bridge between residues 1 and 8
  MISC_FEATURE (1)..(1): N- alpha-acetyl- isoleusine
  THIOETH (2)..(6): Thioether bridge between residues 2 and 8
  MISC_FEATURE (2)..(2): Homocystein
  MISC_FEATURE (6)..(6): N-epsilon-acetyl-lysine
  MISC_FEATURE (8)..(8): Homocystein
XXRGDXYXKKK

SEQ ID NO: 33 - protein, 12 aa, Artificial Sequence
  Integrin-binding Cyclic Peptide 33
  THIOETH (1)..(9): Thioether bridge between residues 1 and 9
  MISC_FEATURE (1)..(1): N- alpha-acetyl- isoleusine
  THIOETH (2)..(6): Thioether bridge between residues 2 and 8
  MISC_FEATURE (2)..(2): Homocystein
  MISC_FEATURE (6)..(6): N-epsilon-acetyl-lysine
  MISC_FEATURE (9)..(9): Homocystein
XXRGDXFRXKKK

SEQ ID NO: 34 - protein, 12 aa, Artificial Sequence
  Integrin-binding Cyclic Peptide 34
  THIOETH (1)..(9): Thioether bridge between residues 1 and 9
  MISC_FEATURE (1)..(1): N- alpha-acetyl- isoleusine
  THIOETH (2)..(6): Thioether bridge between residues 2 and 8
  MISC_FEATURE (2)..(2): Homocystein
  MISC_FEATURE (6)..(6): N-epsilon-acetyl-lysine
  MISC_FEATURE (9)..(9): Homocystein
XXRGDXFAXKKK

SEQ ID NO: 35 - protein, 12 aa, Artificial Sequence
  Integrin-binding Cyclic Peptide 35
  THIOETH (1)..(8): Thioether bridge between residues 1 and 8
  MISC_FEATURE (1)..(1): N- alpha-acetyl- isoleusine
  THIOETH (2)..(6): Thioether bridge between residues 2 and 8
  MISC_FEATURE (2)..(2): Homocystein
  MISC_FEATURE (6)..(6): N-epsilon-acetyl-lysine
  MISC_FEATURE (8)..(8): Homocystein
XXRGDXFXAKKK

SEQ ID NO: 36 - protein, 12 aa, Artificial Sequence
  Integrin-binding Cyclic Peptide 36
  THIOETH (2)..(9): Thioether bridge between residues 2 and 9
  MISC_FEATURE (2)..(2): Homocystein
  THIOETH (3)..(7): Thioether bridge between residues 3 and 7
  MISC_FEATURE (3)..(3): Homocystein
  MISC_FEATURE (7)..(7): N-epsilon-acetyl-lysine
  MISC_FEATURE (9)..(9): N-epsilon-acetyl-lysine
AXXRGDXFXKKK

SEQ ID NO: 37 - protein, 12 aa, Artificial Sequence
  Integrin-binding Cyclic Peptide 37
  THIOETH (4)..(11): Thioether bridge between residues 4 and 11
  MISC_FEATURE (4)..(4): Homocystein
  THIOETH (5)..(9): Thioether bridge between residues 5 and 9
  MISC_FEATURE (5)..(5): Homocystein
  MISC_FEATURE (9)..(9): N-epsilon-acetyl-lysine
  MISC_FEATURE (11)..(11): N-epsilon-acetyl-lysine
KKKXXRGDXFXA

SEQ ID NO: 38 - protein, 11 aa, Artificial Sequence
  Integrin-binding Cyclic Peptide 38
  THIOETH (1)..(8): Thioether bridge between residues 1 and 8
  MISC_FEATURE (1)..(1): N- alpha-acetyl- valine
  MISC_FEATURE (2)..(2): N-delta-acetyl-ornithine
  THIOETH (2)..(6): Thioether bridge between residues 2 and 6
  MISC_FEATURE (6)..(6): Homocystein
  MISC_FEATURE (8)..(8): Homocystein
XXRGDXFXKKK

SEQ ID NO: 39 - protein, 11 aa, Artificial Sequence
  Integrin-binding Cyclic Peptide 39
  THIOETH (1)..(8): Thioether bridge between residues 1 and 8
  MISC_FEATURE (1)..(1): N- alpha-acetyl- aspartic acid
  MISC_FEATURE (2)..(2): N-delta-acetyl-ornithine
  THIOETH (2)..(6): Thioether bridge between residues 2 and 6
  MISC_FEATURE (6)..(6): Homocystein
  MISC_FEATURE (8)..(8): Homocystein
XXRGDXFXKKK

SEQ ID NO: 40 - protein, 11 aa, Artificial Sequence
  Integrin-binding Cyclic Peptide 40
  THIOETH (1)..(8): Thioether bridge between residues 1 and 8
  MISC_FEATURE (1)..(1): N- alpha-acetyl- glutamic acid
  MISC_FEATURE (2)..(2): N-delta-acetyl-ornithine
  THIOETH (2)..(6): Thioether bridge between residues 2 and 6
  MISC_FEATURE (6)..(6): Homocystein
  MISC_FEATURE (8)..(8): Homocystein
XXRGDXFXKKK

SEQ ID NO: 41 - protein, 11 aa, Artificial Sequence
  Integrin-binding Cyclic Peptide 41
  THIOETH (1)..(8): Thioether bridge between residues 1 and 8
  MISC_FEATURE (1)..(1): N- alpha-acetyl- valine
  MISC_FEATURE (2)..(2): Homocystein
  THIOETH (2)..(6): Thioether bridge between residues 2 and 6
  MISC_FEATURE (6)..(6): N-delta-acetyl-ornithine
  MISC_FEATURE (8)..(8): Homocystein
XXRGDXFXKKK

SEQ ID NO: 42 - protein, 11 aa, Artificial Sequence
  Integrin-binding Cyclic Peptide 42
  THIOETH (1)..(8): Thioether bridge between residues 1 and 8
  MISC_FEATURE (1)..(1): N- alpha-acetyl- aspartic acid
  MISC_FEATURE (2)..(2): Homocystein
  THIOETH (2)..(6): Thioether bridge between residues 2 and 6
  MISC_FEATURE (6)..(6): N-delta-acetyl-ornithine
  MISC_FEATURE (8)..(8): Homocystein
XXRGDXFXKKK

SEQ ID NO: 43 - protein, 11 aa, Artificial Sequence
  Integrin-binding Cyclic Peptide 43
  THIOETH (1)..(8): Thioether bridge between residues 1 and 8
  MISC_FEATURE (1)..(1): N- alpha-acetyl- glutamic acid
  MISC_FEATURE (2)..(2): Homocystein
  THIOETH (2)..(6): Thioether bridge between residues 2 and 6
  MISC_FEATURE (6)..(6): N-delta-acetyl-ornithine
  MISC_FEATURE (8)..(8): Homocystein
XXRGDXFXKKK

SEQ ID NO: 44 - protein, 12 aa, Artificial Sequence
  Integrin-binding Cyclic Peptide 44
  THIOETH (1)..(8): Thioether bridge between residues 1 and 8
  MISC_FEATURE (1)..(1): N- alpha-acetyl- valine
  MISC_FEATURE (2)..(2): Homocystein
  THIOETH (2)..(6): Thioether bridge between residues 2 and 6
  MISC_FEATURE (6)..(6): N-epsilon-acetyl-lysine
  MISC_FEATURE (8)..(8): Homocystein
XXRGDXFXAKKK

SEQ ID NO: 45 - protein, 12 aa, Artificial Sequence
  Integrin-binding Cyclic Peptide 45
  THIOETH (1)..(8): Thioether bridge between residues 1 and 8
  MISC_FEATURE (1)..(1): N- alpha-acetyl- aspartic acid
  MISC_FEATURE (2)..(2): Homocystein
  THIOETH (2)..(6): Thioether bridge between residues 2 and 6
  MISC_FEATURE (6)..(6): N-epsilon-acetyl-lysine
  MISC_FEATURE (8)..(8): Homocystein
XXRGDXFXAKKK

SEQ ID NO: 46 - protein, 12 aa, Artificial Sequence
  Integrin-binding Cyclic Peptide 46
  THIOETH (1)..(8): Thioether bridge between residues 1 and 8
  MISC_FEATURE (1)..(1): N- alpha-acetyl- glutamic acid
  MISC_FEATURE (2)..(2): Homocystein
  THIOETH (2)..(6): Thioether bridge between residues 2 and 6
  MISC_FEATURE (6)..(6): N-epsilon-acetyl-lysine
  MISC_FEATURE (8)..(8): Homocystein
XXRGDXFXAKKK

SEQ ID NO: 47 - protein, 12 aa, Artificial Sequence
  Integrin-binding Cyclic Peptide 47
  THIOETH (1)..(8): Thioether bridge between residues 1 and 8
  MISC_FEATURE (1)..(1): N- alpha-acetyl- glutamic acid
  MISC_FEATURE (2)..(2): Homocystein
  THIOETH (2)..(6): Thioether bridge between residues 2 and 6
  MISC_FEATURE (6)..(6): N-delta-acetyl-ornithine
  MISC_FEATURE (8)..(8): Homocystein
XXRGDXFXAKKK

SEQ ID NO: 48 - protein, 11 aa, Artificial Sequence
  Integrin-binding Cyclic Peptide 48
  THIOETH (1)..(8): Thioether bridge between residues 1 and 8
  MISC_FEATURE (1)..(1): N-epsilon-acetyl-lysine
  DISULFID (2)..(6): Disulfid bridge between residues 2 and 6
XCRGDCFCKKK

SEQ ID NO: 49 - protein, 14 aa, Artificial Sequence
  Integrin-binding Cyclic Peptide 49
  DISULFID (2)..(10): Disulfid bridge between residues 2 and 10
  DISULFID (4)..(8): Disulfid bridge between residues 4 and 8
ACDCRGDCFCGKKK